European Patent Application EP 4 299 736 A2, published January 3, 2024. Title: HYDROLASES AND USES THEREOF. Applicant: Vilnius University. The sequence listing filed with the application follows.

SEQUENCE LISTING (41 sequences)

SEQ ID NO: 1 - protein, 132 aa, Metagenomic sequence
MNKEDLLKKAFEAMENAYAPYSNYHVGACALMKDGTTFLGANIENASYGATNCGERSAIFAAYSNGYRADDIEALAIVTDGDRVGAPCGICRQVLSELLNDNTPIYLSNGKETLEKTIDELLPMRFTKEDLL

SEQ ID NO: 2 - protein, 128 aa, Metagenomic sequence
MRHDLVASAMAAREHARAAYSGFKVGAAIRTQDGAIFSGCNIENATLGLTVCAERVALWKALSEGADSFTEIVIATDSDNGGPCGACRQLLWEYCGDIAVRFHSIAGRDQMFRLSELLPHPFDANSLG

SEQ ID NO: 3 - protein, 136 aa, Metagenomic sequence
MKETLCQEARKARENAYCPYSRFMVGAAVLGEDGRIYTGCNIENTSYGMTVCAERTAIFKMVSEGCRKFKALAVAGSTEADGAPCMACRQVMTEFCFDMDVPVYVTCPSGKIYTHTMKEICPYPFMAFDPSEDYGK

SEQ ID NO: 4 - protein, 133 aa, Lachnoclostridium sp.
MRDKLIAEAWEGQKNSYSPYSKFPVGAAVMGADGVIYRGCNIENVSYGLTVCGERNAIFNMVMHGCQTYTALAVVCNGNADAAPCGACRQVMGEFCESLDTPVYICGGEGNLLETTVGELMPYPFLKFDPAKE

SEQ ID NO: 5 - protein, 131 aa, Holdemania filiformis
MYENLVSEAFEAMKSAYAPYSNYHVGACVLCRDGRTFRGVNIENASYGATNCAERSAVFGAYSYGYRKADIAALAIVSDGARIGTPCGICRQVLSELLESDTPIILSNGKETMETTMAELLPMSFGMEDLA

SEQ ID NO: 6 - protein, 133 aa, Solobacterium moorei
MTREELIEEAFKAMENSYAPYSNFHVGAAVLTKDGKVFWGANIENASFGATNCGERSAIFAAYSNGYRKETIEALAIVSDGDRIAAPCGICRQVLSELITGDTPIYLSNRKDEMDTCINELLPYQFTTEDVCR

SEQ ID NO: 7 - protein, 131 aa, Thaumarchaeota archaeon
MNRDDLIKKAREAKEFAYSPYSNFKVGAAILTENGEVFTGCNIENISYGATNCAERTAIFKAISDGNKSFKEIAISSSIAPEKPIFPCGICRQVLAEFNKDMLIHVDGDDKTYKLSELLPAPFDKNQMSNF

SEQ ID NO: 8 - protein, 131 aa, Paenibacillus polymyxa
MKDQLIQKALEARKQAYVPYSNFQVGAAVLGSDGTVYHGCNVENASYGLCNCAERTAIFKMVSEGCRKIDSIAVAADTEGPVSPCGACRQVISEFAHQDTKIYLTNLHGNTEEWTMEQLLPGAFRPADLGK

SEQ ID NO: 9 - protein, 136 aa, Bacillus subtilis
MNRQELITEALKARDMAYAPYSKFQVGAALLTKDGKVYRGCNIENAAYSMCNCAERTALFKAVSEGETEFQMLAVAADTPGPVSPCGACRQVISELCTKDVIVVLTNLQGQIKEMTVEELLPGAFSSEDLHDERKL

SEQ ID NO: 10 - protein, 128 aa, synthetic construct
  REGION 1..128: note = Mutant of 1st sequence
MNKEDLLKKAFEAMENAYAPYSNYHVGACALMKDGTTFLGANIENASYGATNCGERSAIFAAYSNGYRADDIEALAIVTDGDRVGAPCGICRQVLSELLNDNTPIYLSNGKETLEKTIDELLPMRFLL

SEQ ID NO: 11 - protein, 132 aa, synthetic construct
  REGION 1..132: note = Mutant of 1st sequence
MNKEDLLKKAFEAMENAYAPYSNYHVGACALMKDGTTFLGANIENASYGATNCGERSAIFAAYSNGYRADDIEALAIVTDGDRVGAPCGICRQVLSELLNDNTPIYLSNGKETLEKTIDELLPMRATKEDLL

SEQ ID NO: 12 - protein, 132 aa, synthetic construct
  REGION 1..132: note = Mutant of 1st sequence
MNKEDLLKKAFEAMENAYAPYSNYHVGACALMKDGTTFLGANIENASYGATNCGERSAIFAAYSNGYRADDIEALAIVTDGDRVGAPCGICRQVLSELLNDNTPIYLSNGKETLEKTIDELLPMRWTKEDLL

SEQ ID NO: 13 - protein, 132 aa, synthetic construct
  REGION 1..132: note = Mutant of 1st sequence
MNKEDLLKKAFEAMENAYAPYSNYHVGACALMKDGTTFLGANIENASYGATNCGERSAIFAAYSNGYRADDIEALAIVTDGDRVIAPCGICRQVLSELLNDNTPIYLSNGKETLEKTIDELLPMRFTKEDLL

SEQ ID NO: 14 - protein, 132 aa, synthetic construct
  REGION 1..132: note = Mutant of 1st sequence
MNKEDLLKKAFEAMENAYAPYSNYHVGACALMKDGTTFLGANIENASYGAGNCGERSAIFAAYSNGYRADDIEALAIVTDGDRVGAPCGICRQVLSELLNDNTPIYLSNGKETLEKTIDELLPMRFTKEDLL

SEQ ID NO: 15 - protein, 132 aa, synthetic construct
  REGION 1..132: note = Mutant of 1st sequence
MNKEDLLKKAFEAMENAYAPYSNYHVGACALMKDGTTFLGANIENASYGATNCGELSAIFAAYSNGYRADDIEALAIVTDGDRVGAPCGICRQVLSELLNDNTPIYLSNGKETLEKTIDELLPMRFTKEDLL

SEQ ID NO: 16 - protein, 132 aa, synthetic construct
  REGION 1..132: note = Mutant of 1st sequence
MNKEDLLKKAFEAMENAYAPYSNYHVGACALMKDGTTFLGANIENASYGATNCGERSAIFAAYSNGYRADDIEALAIVTDGDQQSAPCGICRQVLSELLNDNTPIYLSNGKETLEKTIDELLPMRFTKEDLL

SEQ ID NO: 17 - protein, 132 aa, synthetic construct
  REGION 1..132: note = Mutant of 1st sequence
MNKEDLLKKAFEAMENAYAPYSNYHVGACALMKDGTTFLGANIENASYGATNCGERSAIFAAYSNGYRADDIEALAIVTDGDSMLAPCGICRQVLSELLNDNTPIYLSNGKETLEKTIDELLPMRFTKEDLL

SEQ ID NO: 18 - protein, 132 aa, synthetic construct
  REGION 1..132: note = Mutant of 1st sequence
MNKEDLLKKAFEAMENAYAPYSNYHVGACALMKDGTTFLGANIENASYGATNCGERSAIFAAYSNGYRADDIEALAIVTDGDHSIAPCGICRQVLSELLNDNTPIYLSNGKETLEKTIDELLPMRFTKEDLL

SEQ ID NO: 19 - protein, 132 aa, synthetic construct
  REGION 1..132: note = Mutant of 1st sequence
MNKEDLLKKAFEAMENAYAPYSNYHVGACALMKDGTTFLGANIENASYGATNCGERSAIFAAYSNGYRADDIEALAIVTDGDRVGAPCGICRQVLSELLNDNTPIYLSNGKETLEKTIDELLPMRFHSSGLL

SEQ ID NO: 20 - protein, 132 aa, synthetic construct
  REGION 1..132: note = Mutant of 1st sequence
MNKEDLLKKAFEAMENAYAPYSNYHVGACALMKDGTTFLGANIENASYGATNCGERSAIFAAYSNGYRADDIEALAIVTDGDRVGAPCGICRQVLSELLNDNTPIYLSNGKETLEKTIDELLPMRFCLYRLL

SEQ ID NO: 21 - protein, 133 aa, synthetic construct
  REGION 1..133: note = Mutant of 4th sequence
MRDKLIAEAWEGQKNSYSPYSKFPVGAAVMGADGVIYRGCNIENVSYGLTVCGERNAIFNMVMHGCQTYTALAVVCNGNADIAPCGACRQVMGEFCESLDTPVYICGGEGNLLETTVGELMPYPFLKFDPAKE

SEQ ID NO: 22 - protein, 131 aa, synthetic construct
  REGION 1..131: note = Mutant of 8th sequence
MKDQLIQKALEARKQAYVPYSNFQVGAAVLGSDGTVYHGCNVENASYGLTNCAERTAIFKMVSEGCRKIDSIAVAADTEGPVSPCGACRQVISEFAHQDTKIYLTNLHGNTEEWTMEQLLPGAFRPADLGK

SEQ ID NO: 23 - protein, 131 aa, synthetic construct
  REGION 1..131: note = Mutant of 8th sequence
MKDQLIQKALEARKQAYVPYSNFQVGAAVLGSDGTVYHGCNVENASYGLCNCAERTAIFKMVSEGCRKIDSIAVAADTEGPLSPCGACRQVISEFAHQDTKIYLTNLHGNTEEWTMEQLLPGAFRPADLGK

SEQ ID NO: 24 - protein, 131 aa, synthetic construct
  REGION 1..131: note = Mutant of 7th sequence
MNRDDLIKKAREAKEFAYSPYSNFKVGAAILTENGEVFTGCNIENISYGATNCAERTAIFKAISDGNKSFKEIAISSSIAPEKPAFPCGICRQVLAEFNKDMLIHVDGDDKTYKLSELLPAPFDKNQMSNF

SEQ ID NO: 25 - protein, 134 aa, Metagenomic sequence
MILLSEAKKKELIELAKEASRKAYAPYSKFKVGVALLAQNGKIYQGCNVENASYSMTICAERNAVFQAVADGNKDFAAIFIYVDSDKSFPPCGACRQVLAEFAGDMLIFIGNRNTVSETTLIEILPERFTLTDE

SEQ ID NO: 26 - protein, 164 aa, Metagenomic sequence
MVTKNISITWTEVNSIEELDKSDRELVLAAREAAQNAHAPYSGFRVGAAVRLASGIIVRGANIENAAFPSGICAERSALSNSASNYPAIKPVALAVAAFTEDGMTQEPVPPCGNCRQVIAEEEFRNNNNIRIILSGENKIQIIEKGGDLLPLQFSKNYLKIKPL

SEQ ID NO: 27 - protein, 152 aa, Metagenomic sequence
MSADERTKNGTPPEQPDDRTLYETAVKMRERSYAPYSRFRVGAALLAKDGMVFTGCNIENASYGACNCAERTAFFKAVSEGVRQFAAIAIAGGPDGAEELDFCPPCGICRQVMEEFCSADFRIILGNTSGELKCLTLAELLPYGFGPGDLDK

SEQ ID NO: 28 - protein, 164 aa, Metagenomic sequence
MKKISITTTISETNSLNDLGIEDQEIISLALSAAGASWSPYSRFAVGAALRLANGVIVTGTNVENAAFPSGICAEHTALSTAASSYPEIAPVAMAITALNKGKQVVTPVAPCGKCRQVIAETENRYKRDIKLFLVGQNKVTIIERGCDLLPLVFSQRDLSSSDE

SEQ ID NO: 29 - protein, 139 aa, Metagenomic sequence
MSKVSDQDLIRLAMEAREYSYSPYSHFMVGAALLAKNGKVYQGCNIENAGYTPSNCAERTAFFKAVSEGVLEFETIAIVAGPKDGELIRTAPCGVCRQVMMEFCEYKTFRVLLAKSPEDYEEWTLEKLLPFGFGPKDLA

SEQ ID NO: 30 - protein, 160 aa, Metagenomic sequence
MTDRRITIDFTEYSSPDEMEPQDRELVAAALRARTGSYSPYSRFRVGAALRLVDGTVVLGANQENVAYPSGLCAERTAMFAAGANHPGVAFDTLAIVGANGDEVCEMPAAPCGACRQVMAEYQRLHGRPLKVILIGTHAIYKFAKVEDLLPLIFDSLKVE

SEQ ID NO: 31 - protein, 145 aa, Metagenomic sequence
MRTKEDFRPLADAAIDASRQSYSPYSQFKVGAAILTADRKVYQGTNVENASYGGTICAERTALVKLVSEERHTMEARAPRTYIEAIAVASNLRGEAVCPCGMCLQFMQEFMSGHEPIILVNRDTRVIEQVLTLQELLPHAFRLLD

SEQ ID NO: 32 - protein, 134 aa, Metagenomic sequence
MTDWTYLIDKAFEARENAYAPYSNFQVGACVETKDGCFIPGANVENAAYGSTICGERNAIFGAYARGYRKEDIKALAIVTGAERISTPCGSCRQVLSELLEPDTPIVLCNRKDTVVTNIAELLPGAFGAEDLAK

SEQ ID NO: 33 - protein, 166 aa, Metagenomic sequence
MDLERSRTLFQTIGGEPINNDLVVTMIAQAREARAFSYAPYSNYNVGCAALLERDGKRSIFRGTNIENAAYWPTMCAERSAIFSAASLGFRKLLAVAVVGDRDDTSLVTPCGGCRQVMNEFGNALTLIIMAKEDDTVELRTLGQLLPEAFGPSNLGMNPQNYMAKK

SEQ ID NO: 34 - protein, 154 aa, Metagenomic sequence
MTEKKITTKVRVYSYNELTEEQKKLVDLAREATSHSYSPYSNFKVGAALMLDNGEVFIGANQENAAFAGICGERAALYAAGAKHPGVPVKSVAITSFTRDAFVEEPTAPCGVCRQAFLEFEKNGHPIELILAGKEKIYILDSFKDTMPLSFTEF

SEQ ID NO: 35 - protein, 139 aa, Metagenomic sequence
MNQLTQQEMDLLLDKAQEARDHSYAPYSKYNVGAALMTADGQIYQGCNIENAGFTPTVCAERTAFFKAVYDGHRAFRAIAVIATGEELGFPCGVCRQVMAEFCDRDFIIVTANRDRTKVDVSDFETLLPHSFGPKDLGV

SEQ ID NO: 36 - protein, 136 aa, Metagenomic sequence
MTNVTPEDAKFLIDLANQARERAYAPYSNYHVGAALRTKSGRIFTGVNVENAAYPTTMCAERVAIYKAVSEGELEFDVIAVVTSNGGSPCGGCRQVMAEFGLETVVLIGNGAGEILEETTVNGLLPGAFTPAHLKS

SEQ ID NO: 37 - protein, 132 aa, Metagenomic sequence
MTETDKKLIAEAKRVREFAYCPYSKFAVGAAVLGASGEIYGGCNIENASFSVTNCAERTAIFKAVSAGEDDILAIAVVAEGVNPVPPCGACRQVIAEFNIPHILMANLADEVKEMTLEELLPGAFSAEDING

SEQ ID NO: 38 - protein, 135 aa, Metagenomic sequence
MDAGLLMQEAIKARTRAYIPYSKFGVGAALLDSRGQVHLGCNVENAAYGPTNCAERTALFRAIADGHEAGSFQAIAIVADTDGPCTPCGVCRQVLVELCKPDMKVIMGNMKGDIKETTVSELLPGAFGPWDLNKQ

SEQ ID NO: 39 - protein, 135 aa, Metagenomic sequence
MDAGLLMQEAIKARMRAYIPYSTFGVGAALLDSHGEVHLGCNVENAAYGPTNCAERTALFRAIADGHEAGSFQAIAIVADTEGPCTPCGVCRQVLVELCKPDMKVIMGNMKGDIKETTVIELLPGAFGPWDLNKQ

SEQ ID NO: 40 - protein, 132 aa, Metagenomic sequence
MNKQELISEAVKARDFAYVPYSKFKVGAALLSHDGKVYGGCNIENAAYGMCNCAERTALFKAYSEGITSFQMLAVVADTDRPVSPCGACRQVISELCAPDMPVILTNLKGHIYETTVNELLPGAFSPEDLND

SEQ ID NO: 41 - protein, 133 aa, Metagenomic sequence
MIAAASRAREFSYAPYSNFTVGAALITKSGKVFTGCNVESVSYSPTTCAERVAILKAVSEGERSFEMIVVIGGPRVGESKAKGYSGPCGVCRQMIYEFGKDIQIIIANSLDEYYVHDISELFPLGFGPDHLLG